European Patent Application EP 4 174 180 A1, published May 3, 2023. Title: Polynucleotide, polynucleotide set, detection method for Porphyromonas gingivalis, evaluation method for susceptibility of periodontal disease, detection kit for Porphyromonas gingivalis, and evaluation kit for susceptibility of periodontal disease. Applicant: Mitsui Chemicals, Inc. The sequence listing filed with the application follows.

SEQUENCE LISTING (18 sequences)

SEQ ID NO: 1 - DNA, 21 bp, Artificial Sequence
  primer
aagctgacaaagcatgatggt

SEQ ID NO: 2 - DNA, 20 bp, Artificial Sequence
  primer
aagctgacaaagcatgatgg

SEQ ID NO: 3 - DNA, 18 bp, Artificial Sequence
  primer
agctgacaaagcatgatg

SEQ ID NO: 4 - DNA, 24 bp, Artificial Sequence
  primer
tattcttaggcgtataaccattgt

SEQ ID NO: 5 - DNA, 25 bp, Artificial Sequence
  primer
atagttgttgctgttgaagtttacc

SEQ ID NO: 6 - DNA, 27 bp, Artificial Sequence
  primer
attttattcttaggcgtataaccattg

SEQ ID NO: 7 - DNA, 23 bp, Artificial Sequence
  primer
agttgttgctgttgaagtttacc

SEQ ID NO: 8 - DNA, 29 bp, Artificial Sequence
  primer
ctcaattttattcttaggcgtataaccat

SEQ ID NO: 9 - DNA, 21 bp, Artificial Sequence
  primer
tattcttaggcgtataaccat

SEQ ID NO: 10 - DNA, 20 bp, Artificial Sequence
  primer
gcatgatggtactcctttga

SEQ ID NO: 11 - DNA, 20 bp, Artificial Sequence
  primer
ctgaccaacgagaacccact

SEQ ID NO: 12 - DNA, 22 bp, Artificial Sequence
  primer
acaactatacttatgacaatgg

SEQ ID NO: 13 - DNA, 22 bp, Artificial Sequence
  primer
aaccccgctccctgtattccga

SEQ ID NO: 14 - DNA, 20 bp, Artificial Sequence
  primer
tagcttgctaaggttgatgg

SEQ ID NO: 15 - DNA, 20 bp, Artificial Sequence
  primer
caagtgtatgcggttttagt

SEQ ID NO: 16 - DNA, 20 bp, Artificial Sequence
  TaqMan probe
  misc_feature (1)..(1): n is adenine modified by FAM
  misc_feature (20)..(20): n is thymine modified by NFQ and MGB
ncttcaacagcaacaactan

SEQ ID NO: 17 - DNA, 20 bp, Artificial Sequence
  TaqMan probe
  misc_feature (1)..(1): n is adenine modified by HEX
  misc_feature (20)..(20): n is thymine modified by MGB and EG
ntagttgttgctgttgaagn

SEQ ID NO: 18 - DNA, 22 bp, Artificial Sequence
  TaqMan probe
  misc_feature (1)..(1): n is cytosine modified by HEX
  misc_feature (22)..(22): n is thymine modified by MGB and EQ
nctacgacctattatcctgtan